European Patent Application EP 4 785 960 A1, published August 5, 2026. Title: GLP-1 ANTIBODY CONJUGATES. Applicant: SIXPEAKS BIO AG. Application EP. The sequence listing filed with the application follows.

SEQUENCE LISTING (67 sequences)

SEQ ID NO: 1 - protein, 47 aa, synthetic construct
  MOD_RES 2: note = Aib
  MOD_RES 47: note = Lysine is linked with acetylbromide
HXEGTFTSDYSSYLEEQAAKEFIAWLVKGGGGGGGSGGGGSGGGGSK

SEQ ID NO: 2 - protein, 47 aa, synthetic construct
  MOD_RES 2: note = Aib
  MOD_RES 47: note = Lysine is linked with acetylbromide
HXEGTFTSDVSSYLEGQAAKEFIAWLVKGGGGGGGSGGGGSGGGGSK

SEQ ID NO: 3 - protein, 32 aa, synthetic construct
  MOD_RES 2: note = Aib
  SITE 32: note = The side chain of the lysine is linked via an amide linkage to SEQ ID NO:62
HXEGTFTSDVSSYLEEQAAKEFIAWLVKGGGK

SEQ ID NO: 4 - protein, 31 aa, synthetic construct
  MOD_RES 2: note = Aib
  SITE 20: note = The side chain of the lysine is linked via an amide linkage to SEQ ID NO:64
HXEGTFTSDVSSYLEGQAAKEFIAWLVKGGG

SEQ ID NO: 5 - protein, 47 aa, synthetic construct
  MOD_RES 2: note = Aib
  MOD_RES 16: note = Aib
  SITE 13: note = D-Tyrosine
  SITE 14: note = D-Leucine
  MOD_RES 47: note = Lysine is linked with acetylbromide
HXEGTFTSDVSSYLEXQAAKEFIAWLVKGGGGGGGSGGGGSGGGGSK

SEQ ID NO: 6 - protein, 42 aa, synthetic construct
  MOD_RES 2: note = Aib
  MOD_RES 32: note = bAla
  MOD_RES 34: note = bAla
  MOD_RES 36: note = bAla
  MOD_RES 38: note = bAla
  MOD_RES 40: note = bAla
  MOD_RES 33: note = Gamma-glutamic acid
  MOD_RES 35: note = Gamma-glutamic acid
  MOD_RES 37: note = Gamma-glutamic acid
  MOD_RES 39: note = Gamma-glutamic acid
  MOD_RES 41: note = Gamma-glutamic acid
  MOD_RES 42: note = Lysine is linked with acetylbromide
HXEGTFTSDYSSYLEEQAAKEFIAWLVKGGGXXXXXXXXXXK

SEQ ID NO: 7 - protein, 42 aa, synthetic construct
  MOD_RES 33: note = Gamma-glutamic acid
  MOD_RES 35: note = Gamma-glutamic acid
  MOD_RES 37: note = Gamma-glutamic acid
  MOD_RES 39: note = Gamma-glutamic acid
  MOD_RES 41: note = Gamma-glutamic acid
  MOD_RES 32: note = bAla
  MOD_RES 34: note = bAla
  MOD_RES 36: note = bAla
  MOD_RES 38: note = bAla
  MOD_RES 40: note = bAla
  MOD_RES 2: note = Aib
  MOD_RES 42: note = Lysine is linked with acetylbromide
HXEGTFTSDVSSYLEGQAAKEFIAWLVKGGGXXXXXXXXXXK

SEQ ID NO: 8 - protein, 32 aa, synthetic construct; identical to SEQ ID NO: 3
  MOD_RES 2: note = Aib
  SITE 32: note = The side chain of the lysine is linked via an amide linkage to sequence gamma-E beta-A gamma-E beta-A gamma-E beta-A gamma-E beta-A gamma-E beta-AAcBr

SEQ ID NO: 9 - protein, 32 aa, synthetic construct
  MOD_RES 32: note = Lysine is linked with 1-Amino-3,6,9,12-tetraoxapentadecan-15-oic acid-CAS 581065-95-4-acetylbromide
HGEGTFTSDVSSYLEEQAAKEFIAWLVKGGGK

SEQ ID NO: 10 - protein, 32 aa, synthetic construct; identical to SEQ ID NO: 9
  SITE 32: note = The side chain of the lysine is linked via an amide linkage to SEQ ID NO:65

SEQ ID NO: 11 - protein, 31 aa, synthetic construct
  MOD_RES 2: note = Aib
  MOD_RES 20: note = Lysine is linked with 1-Amino-3,6,9,12-tetraoxapentadecan-15-oic acid-CAS 581065-95-4-acetylbromide
HXEGTFTSDVSSYLEGQAAKEFIAWLVRGRG

SEQ ID NO: 12 - protein, 31 aa, synthetic construct; identical to SEQ ID NO: 11
  MOD_RES 2: note = Aib
  SITE 20: note = The side chain of the lysine is linked via an amide linkage to SEQ ID NO:66

SEQ ID NO: 13 - protein, 32 aa, synthetic construct
  MOD_RES 2: note = Aib
  MOD_RES 32: note = Lysine is linked with 1-Amino-3,6,9,12-tetraoxapentadecan-15-oic acid-CAS 581065-95-4-acetylbromide
HXEGTFTSDVSSYLEGQAAKEFIAWLVRGRGK

SEQ ID NO: 14 - protein, 32 aa, synthetic construct; identical to SEQ ID NO: 13
  MOD_RES 2: note = Aib
  SITE 32: note = The side chain of the lysine is linked via an amide linkage to SEQ ID NO:67

SEQ ID NO: 15 - protein, 32 aa, synthetic construct; identical to SEQ ID NO: 3
  MOD_RES 2: note = Aib
  SITE 32: note = The side chain of the lysine is linked via an amide linkage to SEQ ID NO:63

SEQ ID NO: 16 - protein, 445 aa, synthetic construct
QVQLVQSGAEVKKPGASVKVSCKASGYTFTSSYINWVRQAPGQGLEWMGTINPVSGSTSYAQKFQGRVTMTRDTSISTAYMELSRLRSDDTAVYYCARGGWFDYWGQGTLVTVSSASTKGPSVFPLAPSSKSTSGGTAALGCLVKDYFPEPVTVSWNSGALTSGVHTFPAVLQSSGLYSLSSVVTVPSSSLGTQTYICNVNHKPSNTKVDKKVEPKSCDKTHTCPPCPAPEAAGGPSVFLFPPKPKDTLYITREPEVTCVVVDVSHEDPCVKFNWYVDGVEVHNAKTKPREEQYNSTYRVVSVLTVLHQDWLNGKEYKCKVSNKALAAPIEKTISKAKGQPREPQVYTLPPSREEMTKNQVSLTCLVKGFYPSDIAVEWESNGQPENNYKTTPPVLDSDGSFFLYSKLTVDKSRWQQGNVFSCSVMHEALHNHYTQKSLSLSPGK

SEQ ID NO: 17 - protein, 217 aa, synthetic construct
QSALTQPASVSGSPGQSITISCTGTSSDVGSYNYVNWYQQHPGKAPKLMIYGVSKRPSGVSNRFSGSKSGNTASLTISGLQAEDEADYYCGTFAGGSYYGVFGGGTKLTVLGQPKAAPSVTLFPPSSEELQANKATLVCLISDFYPGAVTVAWKADSSPVKAGVETTTPSKQSNNKYAASSYLSLTPEQWKSHRSYSCQVTHEGSTVEKTVAPTECS

SEQ ID NO: 18 - protein, 115 aa, synthetic construct [sequence omitted]

SEQ ID NO: 19 - protein, 111 aa, synthetic construct [sequence omitted]

SEQ ID NO: 20 - protein, 5 aa, synthetic construct
SSYIN

SEQ ID NO: 21 - protein, 17 aa, synthetic construct
TINPVSGSTSYAQKFQG

SEQ ID NO: 22 - protein, 6 aa, synthetic construct
GGWFDY

SEQ ID NO: 23 - protein, 14 aa, synthetic construct
TGTSSDVGSYNYVN

SEQ ID NO: 24 - protein, 7 aa, synthetic construct
GVSKRPS

SEQ ID NO: 25 - protein, 11 aa, synthetic construct
GTFAGGSYYGV

SEQ ID NO: 26 - protein, 445 aa, synthetic construct
QVQLVQSGAEVKKPGSSVKVSCKASGYTFTSSYINWVRQAPGQGLEWMGTINAVSGSTSYAQKFQGRVTITADTSTSTAYMELSSLRSEDTAVYYCARGGWFDYWGQGTLVTVSSASTKGPSVFPLAPSSKSTSGGTAALGCLVKDYFPEPVTVSWNSGALTSGVHTFPAVLQSSGLYSLSSVVTVPSSSLGTQTYICNVNHKPSNTKVDKKVEPKSCDKTHTCPPCPAPEAAGGPSVFLFPPKPKDTLMISRTPEVTCVVVDVSHEDPCVKFNWYVDGVEVHNAKTKPREEQYNSTYRVVSVLTVLHQDWLNGKEYKCKVSNKALAAPIEKTISKAKGQPREPQVYTLPPSREEMTKNQVSLTCLVKGFYPSDIAVEWESNGQPENNYKTTPPVLDSDGSFFLYSKLTVDKSRWQQGNVFSCSVMHEALHNHYTQKSLSLSPGK

SEQ ID NO: 27 - protein, 217 aa, synthetic construct
QSALTQPRSVSGSPGQSVTISCTGTSSDVGSKNYVNWYQQHPGKAPKLMIYGVSKRESGVPDRFSGSKSGNTASLTISGLQAEDEADYYCGTFAGGKYYGVFGGGTKLTVLGQPKAAPSVTLFPPSSEELQANKATLVCLISDFYPGAVTVAWKADSSPVKAGVETTTPSKQSNNKYAASSYLSLTPEQWKSHRSYSCQVTHEGSTVEKTVAPTECS

SEQ ID NO: 28 - protein, 115 aa, synthetic construct
QVQLVQSGAEVKKPGSSVKVSCKASGYTFTSSYINWVRQAPGQGLEWMGTINAVSGSTSYAQKFQGRVTITADTSTSTAYMELSSLRSEDTAVYYCARGGWFDYWGQGTLVTVSS

SEQ ID NO: 29 - protein, 111 aa, synthetic construct
QSALTQPRSVSGSPGQSVTISCTGTSSDVGSKNYVNWYQQHPGKAPKLMIYGVSKRESGVPDRFSGSKSGNTASLTISGLQAEDEADYYCGTFAGGKYYGVFGGGTKLTVL

SEQ ID NO: 30 - protein, 17 aa, synthetic construct
TINAVSGSTSYAQKFQG

SEQ ID NO: 31 - protein, 14 aa, synthetic construct
TGTSSDVGSKNYVN

SEQ ID NO: 32 - protein, 7 aa, synthetic construct
GVSKRES

SEQ ID NO: 33 - protein, 11 aa, synthetic construct
GTFAGGKYYGV

SEQ ID NO: 34 - protein, 445 aa, synthetic construct
QVQLVQSGAEVKKPGSSVKVSCKASGYTFTSSYINWVRQAPGQGLEWMGTINAVSGSTSYAQKFQGRVTITADTSTSTAYMELSSLRSEDTAVYYCARGGWFDYWGQGTLVTVSSAKTTAPSVYPLAPVCGDTTGSSVTLGCLVKGYFPEPVTLTWNSGSLSSGVHTFPAVLQSDLYTLSSSVTVTSSTWPSQSITCNVAHPASSTKVDKKIEPRGPTIKPCPPCKCPAPNAAGGPSVFIFPPKIKDVLMISLSPIVTCVVVDVSEDDPCVQISWFVNNVEVHTAQTQTHREDYNSTLRVVSALPIQHQDWMSGKEFKCKVNNKDLAAPIERTISKPKGSVRAPQVYVLPPPEEEMTKKQVTLTCMVTDFMPEDIYVEWTNNGKTELNYKNTEPVLDSDGSYFMYSKLRVEKKNWVERNSYSCSVVHEGLHNHHTTKSFSRTPGK

SEQ ID NO: 35 - protein, 217 aa, synthetic construct
QSALTQPRSVSGSPGQSVTISCTGTSSDVGSANYVNWYQQHPGKAPKPMIYGVSRRPSGVPDRFSGSKSGNTASLTISGLQAEDEADYYCGTFAGGKYYGVFGGGTKLTVLGQPKAAPSVTLFPPSSEELQANKATLVCLISDFYPGAVTVAWKADSSPVKAGVETTTPSKQSNNKYAASSYLSLTPEQWKSHRSYSCQVTHEGSTVEKTVAPTECS

SEQ ID NO: 36 - protein, 111 aa, synthetic construct
QSALTQPRSVSGSPGQSVTISCTGTSSDVGSANYVNWYQQHPGKAPKPMIYGVSRRPSGVPDRFSGSKSGNTASLTISGLQAEDEADYYCGTFAGGKYYGVFGGGTKLTVL

SEQ ID NO: 37 - protein, 14 aa, synthetic construct
TGTSSDVGSANYVN

SEQ ID NO: 38 - protein, 7 aa, synthetic construct
GVSRRPS

SEQ ID NO: 39 - protein, 445 aa, synthetic construct
QVQLVQSGAEVRKPGSSVKVSCKASGYTFTSSYINWVRQAPGQGLEWMGTINPVSGSTSYAQKFQGRVTITADTSTSTAYMELSSLRSEDTAVYYCARGGWFDYWGQGTLVTVSSAKTTAPSVYPLAPVCGDTTGSSVTLGCLVKGYFPEPVTLTWNSGSLSSGVHTFPAVLQSDLYTLSSSVTVTSSTWPSQSITCNVAHPASSTKVDKKIEPRGPTIKPCPPCKCPAPNAAGGPSVFIFPPKIKDVLMISLSPIVTCVVVDVSEDDPCVQISWFVNNVEVHTAQTQTHREDYNSTLRVVSALPIQHQDWMSGKEFKCKVNNKDLAAPIERTISKPKGSVRAPQVYVLPPPEEEMTKKQVTLTCMVTDFMPEDIYVEWTNNGKTELNYKNTEPVLDSDGSYFMYSKLRVEKKNWVERNSYSCSVVHEGLHNHHTTKSFSRTPGK

SEQ ID NO: 40 - protein, 217 aa, synthetic construct
QSALTQPRSVSGSPGQSVTISCTGTSSDVGSYNRVNWYQQHPGKAPKLMIYGVSKRESGVPDRFSGSKSGNTASLTISGLQAEDEADYYCGTFAGGRYYGVFGGGTKLTVLGQPKAAPSVTLFPPSSEELQANKATLVCLISDFYPGAVTVAWKADSSPVKAGVETTTPSKQSNNKYAASSYLSLTPEQWKSHRSYSCQVTHEGSTVEKTVAPTECS

SEQ ID NO: 41 - protein, 115 aa, synthetic construct
QVQLVQSGAEVRKPGSSVKVSCKASGYTFTSSYINWVRQAPGQGLEWMGTINPVSGSTSYAQKFQGRVTITADTSTSTAYMELSSLRSEDTAVYYCARGGWFDYWGQGTLVTVSS

SEQ ID NO: 42 - protein, 111 aa, synthetic construct
QSALTQPRSVSGSPGQSVTISCTGTSSDVGSYNRVNWYQQHPGKAPKLMIYGVSKRESGVPDRFSGSKSGNTASLTISGLQAEDEADYYCGTFAGGRYYGVFGGGTKLTVL

SEQ ID NO: 43 - protein, 14 aa, synthetic construct
TGTSSDVGSYNRVN

SEQ ID NO: 44 - protein, 11 aa, synthetic construct
GTFAGGRYYGV

SEQ ID NO: 45 - protein, 217 aa, synthetic construct
QSALTQPRSVSGSPGQSVTISCTGTSSDVGSKNYVNWYQQHPGKAPKLMIYGVSKRESGVPDRFSGSKSGNTASLTISGLQAEDEADYYCGTFAGGKYYGVFGGGTKLTVLGQPKSSPSVTLFPPSSEELETNKATLVCTITDFYPGVVTVDWKVDGTPVTQGMETTQPSKQSNNKYMASSYLTLTARAWERHSSYSCQVTHEGHTVEKSLSRADCS

SEQ ID NO: 46 - protein, 217 aa, synthetic construct
QSALTQPRSVSGSPGQSVTISCTGTSSDVGSANYVNWYQQHPGKAPKPMIYGVSRRPSGVPDRFSGSKSGNTASLTISGLQAEDEADYYCGTFAGGKYYGVFGGGTKLTVLGQPKSSPSVTLFPPSSEELETNKATLVCTITDFYPGVVTVDWKVDGTPVTQGMETTQPSKQSNNKYMASSYLTLTARAWERHSSYSCQVTHEGHTVEKSLSRADCS

SEQ ID NO: 47 - protein, 217 aa, synthetic construct
QSALTQPRSVSGSPGQSVTISCTGTSSDVGSYNRVNWYQQHPGKAPKLMIYGVSKRESGVPDRFSGSKSGNTASLTISGLQAEDEADYYCGTFAGGRYYGVFGGGTKLTVLGQPKSSPSVTLFPPSSEELETNKATLVCTITDFYPGVVTVDWKVDGTPVTQGMETTQPSKQSNNKYMASSYLTLTARAWERHSSYSCQVTHEGHTVEKSLSRADCS

SEQ ID NO: 48 - protein, 458 aa, synthetic construct
QVQLQQSGPGLVKPSQTLSLTCAISGDSVSSNSAAWSWIRQSPGRGLEWLGRIYYRSKWYNDYAVSVKSRITINPDTSKNQFSLQLNSVTPEDTAVYYCARLDHRYHEDTVYPGMDVWGQGTLVTVSSAKTTAPSVYPLAPVCGDTTGSSVTLGCLVKGYFPEPVTLTWNSGSLSSGVHTFPAVLQSDLYTLSSSVTVTSSTWPSQSITCNVAHPASSTKVDKKIEPRGPTIKPCPPCKCPAPNAAGGPSVFIFPPKIKDVLMISLSPIVTCVVVDVSEDDPCVQISWFVNNVEVHTAQTQTHREDYNSTLRVVSALPIQHQDWMSGKEFKCKVNNKDLAAPIERTISKPKGSVRAPQVYVLPPPEEEMTKKQVTLTCMVTDFMPEDIYVEWTNNGKTELNYKNTEPVLDSDGSYFMYSKLRVEKKNWVERNSYSCSVVHEGLHNHHTTKSFSRTPGK

SEQ ID NO: 49 - protein, 213 aa, synthetic construct
DIELTQPPSVSVAPGQTARISCSGDNLPAYTVTWYQQKPGQAPVLVIYDDSDRPSGIPERFSGSNSGNTATLTISGTQAEDEADYYCASWDPSSGVVFGGGTKLTVLGQPKSSPSVTLFPPSSEELETNKATLVCTITDFYPGVVTVDWKVDGTPVTQGMETTQPSKQSNNKYMASSYLTLTARAWERHSSYSCQVTHEGHTVEKSLSRADCS

SEQ ID NO: 50 - protein, 128 aa, synthetic construct
QVQLQQSGPGLVKPSQTLSLTCAISGDSVSSNSAAWSWIRQSPGRGLEWLGRIYYRSKWYNDYAVSVKSRITINPDTSKNQFSLQLNSVTPEDTAVYYCARLDHRYHEDTVYPGMDVWGQGTLVTVSS

SEQ ID NO: 51 - protein, 107 aa, synthetic construct
DIELTQPPSVSVAPGQTARISCSGDNLPAYTVTWYQQKPGQAPVLVIYDDSDRPSGIPERFSGSNSGNTATLTISGTQAEDEADYYCASWDPSSGVVFGGGTKLTVL

SEQ ID NO: 52 - protein, 7 aa, synthetic construct
SNSAAWS

SEQ ID NO: 53 - protein, 18 aa, synthetic construct
RIYYRSKWYNDYAVSVKS

SEQ ID NO: 54 - protein, 16 aa, synthetic construct
LDHRYHEDTVYPGMDV

SEQ ID NO: 55 - protein, 11 aa, synthetic construct
SGDNLPAYTVT

SEQ ID NO: 56 - protein, 7 aa, synthetic construct
DDSDRPS

SEQ ID NO: 57 - protein, 10 aa, synthetic construct
ASWDPSSGVV

SEQ ID NO: 58 - protein, 513 aa, Homo sapiens
MGAAAKLAFAVFLISCSSGAILGRSETQECLFFNANWEKDRTNQTGVEPCYGDKDKRRHCFATWKNISGSIEIVKQGCWLDDINCYDRTDCVEKKDSPEVYFCCCEGNMCNEKFSYFPEMEVTQPTSNPVTPKPPYYNILLYSLVPLMLIAGIVICAFWVYRHHKMAYPPVLVPTQDPGPPPPSPLLGLKPLQLLEVKARGRFGCVWKAQLLNEYVAVKIFPIQDKQSWQNEYEVYSLPGMKHENILQFIGAEKRGTSVDVDLWLITAFHEKGSLSDFLKANVVSWNELCHIAETMARGLAYLHEDIPGLKDGHKPAISHRDIKSKNVLLKNNLTACIADFGLALKFEAGKSAGDTHGQVGTRRYMAPEVLEGAINFQRDAFLRIDMYAMGLVLWELASRCTAADGPVDEYMLPFEEEIGQHPSLEDMQEVVVHKKKRPVLRDYWQKHAGMAMLCETIEECWDHDAEARLSAGCVGERITQMQRLTNIITTEDIVTVVTMVTNVDFPPKESSL

SEQ ID NO: 59 - protein, 512 aa, Homo sapiens
MTAPWVALALLWGSLCAGSGRGEAETRECIYYNANWELERTNQSGLERCEGEQDKRLHCYASWRNSSGTIELVKKGCWLDDFNCYDRQECVATEENPQVYFCCCEGNFCNERFTHLPEAGGPEVTYEPPPTAPTLLTVLAYSLLPIGGLSLIVLLAFWMYRHRKPPYGHVDIHEDPGPPPPSPLVGLKPLQLLEIKARGRFGCVWKAQLMNDFVAVKIFPLQDKQSWQSEREIFSTPGMKHENLLQFIAAEKRGSNLEVELWLITAFHDKGSLTDYLKGNIITWNELCHVAETMSRGLSYLHEDVPWCRGEGHKPSIAHRDFKSKNVLLKSDLTAVLADFGLAVRFEPGKPPGDTHGQVGTRRYMAPEVLEGAINFQRDAFLRIDMYAMGLVLWELVSRCKAADGPVDEYMLPFEEEIGQHPSLEELQEVVVHKKMRPTIKDHWLKHPGLAQLCVTIEECWDHDAEARLSAGCVEERVSLIRRSVNGTTSDCLVSLVTSVTNVDLPPKESSI

SEQ ID NO: 60 - protein, 445 aa, synthetic construct; identical to SEQ ID NO: 34

SEQ ID NO: 61 - protein, 115 aa, synthetic construct; identical to SEQ ID NO: 28

SEQ ID NO: 62 - protein, 15 aa, synthetic construct
  SITE 1: note = The side chain of the glycine is linked via an amide linkage to SEQ ID NO:3
  MOD_RES 15: note = Serine is linked with acetylbromide
GGGGSGGGGSGGGGS

SEQ ID NO: 63 - protein, 18 aa, synthetic construct
  SITE 1: note = The side chain of the alanine is linked via an amide linkage to SEQ ID NO:15
  MOD_RES 18: note = Alanine is linked with acetylbromide
AAAKAAAEAAAKAAAEAA

SEQ ID NO: 64 - protein, 15 aa, synthetic construct
  MOD_RES 15: note = Serine is linked with acetylbromide
  SITE 1: note = The side chain of the glycine is linked via an amide linkage to SEQ ID NO:4
GGGGSGGGGSGGGGS

SEQ ID NO: 65 - protein, 15 aa, synthetic construct
  MOD_RES 15: note = Serine is linked with acetylbromide
  SITE 1: note = The side chain of the glycine is linked via an amide linkage to SEQ ID NO:10
GGGGSGGGGSGGGGS

SEQ ID NO: 66 - protein, 15 aa, synthetic construct
  MOD_RES 15: note = Serine is linked with acetylbromide
  SITE 1: note = The side chain of the glycine is linked via an amide linkage to SEQ ID NO:12
GGGGSGGGGSGGGGS

SEQ ID NO: 67 - protein, 15 aa, synthetic construct
  MOD_RES 15: note = Serine is linked with acetylbromide
  SITE 1: note = The side chain of the glycine is linked via an amide linkage to SEQ ID NO:14
GGGGSGGGGSGGGGS